European Patent Specification EP 4 103 160 B1, published June 26, 2024. Title: NANOPARTICLES ENCAPSULATING SMALL MOLECULES. Applicant: ETH Zurich. The sequence listing filed with the application follows.

SEQUENCE LISTING (27 sequences)

SEQ ID NO: 1 - protein, 186 aa, Artificial Sequence
  Synthetic sequence
  MISC_FEATURE (2)..(2): Any amino acid
  MISC_FEATURE (11)..(11): At least 3 of the X amino acids at positions 11, 39, 66, 103,, 130, and 163  are independently of each other a positively charged amino acid.
  MISC_FEATURE (28)..(28): Any amino acid
  MISC_FEATURE (30)..(30): Any amino acid
  MISC_FEATURE (39)..(39): At least 3 of the X amino acids at positions 11, 39, 66, 103,, 130, and 163  are independently of each other a positively charged amino acid.
  MISC_FEATURE (51)..(51): Any amino acid
  MISC_FEATURE (54)..(54): Any amino acid
  MISC_FEATURE (55)..(55): Any amino acid
  MISC_FEATURE (58)..(58): Any amino acid
  MISC_FEATURE (62)..(62): Any amino acid
  MISC_FEATURE (66)..(66): At least 3 of the X amino acids at positions 11, 39, 66, 103,, 130, and 163  are independently of each other a positively charged amino acid.
  MISC_FEATURE (76)..(76): Any amino acid
  MISC_FEATURE (86)..(86): Any amino acid
  MISC_FEATURE (88)..(88): Any amino acid
  MISC_FEATURE (90)..(90): Any amino acid
  MISC_FEATURE (92)..(92): Any amino acid
  MISC_FEATURE (93)..(93): Any amino acid
  MISC_FEATURE (94)..(94): Any amino acid
  MISC_FEATURE (103)..(103): At least 3 of the X amino acids at positions 11, 39, 66, 103,, 130, and 163  are independently of each other a positively charged amino acid.
  MISC_FEATURE (114)..(114): Any amino acid
  MISC_FEATURE (117)..(117): Any amino acid
  MISC_FEATURE (120)..(120): Any amino acid
  MISC_FEATURE (130)..(130): At least 3 of the X amino acids at positions 11, 39, 66, 103,, 130, and 163  are independently of each other a positively charged amino acid.
  MISC_FEATURE (163)..(163): At least 3 of the X amino acids at positions 11, 39, 66, 103,, 130, and 163  are independently of each other a positively charged amino acid.
  MISC_FEATURE (172)..(172): Any amino acid
  MISC_FEATURE (175)..(175): Any amino acid
  MISC_FEATURE (179)..(179): Any amino acid
  MISC_FEATURE (183)..(183): Any amino acid
  MISC_FEATURE (185)..(185): Any amino acid
MXQAIGILELXSIAAGMELGDAMLKSAXVXLLVSKTISXGKFLLMLGGDIXAIXXAIXTGTXQAGXLLVDSLVLAXIHPSVLPAIXGXNXVXXXQAVGIVETXSVAACISAADXAVXGSXVTLVRVHMAXGIGGKCYMVVAGDVSDVALAVTVASSSAGAYGXLVYASLIPXPHXAMWXQMVXGXE

SEQ ID NO: 2 - protein, 192 aa, Artificial Sequence
  Synthetic sequence
MSQAIGILELRSIAAGMELGDAMLKSANVDLLVSKTISRGKFLLMLGGDIGAIQQAIETGTSQAGRLLVDSLVLANIHPSVLPAISGLNSVDKRQAVGIVETRSVAACISAADRAVKGSNVTLVRVHMARGIGGKCYMVVAGDVSDVALAVTVASSSAGAYGRLVYASLIPRPHEAMWRQMVEGLEHHHHHH

SEQ ID NO: 3 - protein, 188 aa, Artificial Sequence
  Synthetic sequence
MSQAIGILELRSIAAGMELGDAMLKSANVDLLVSKTISRGKFLLMLGGDIGAIQQAIETGTSQAGRLLVDSLVLANIHPSVLPAISGLNSVDKRQAVGIVETRSVAACISAADRAVKGSNVTLVRVHMARGIGGKCYMVVAGDVSDVALAVTVASSSAGAYGRLVYASLIPRPHEAMWRQMVEGLEGS

SEQ ID NO: 4 - protein, 192 aa, Artificial Sequence
  Synthetic sequence
MSQAIGILELRSIAAGMELGDAMLKSANVDLLVSKTISRGKFLLMLGGDIGAIQQAIETGTSQAGRLLVDSLVLANIHPSVLPAISGLNSVDCRQAVGIVETRSVAACISAADRAVKGSNVTLVRVHMARGIGGKCYMVVAGDVSDVALAVTVASSSAGAYGRLVYASLIPRPHEAMWRQMVEGLEHHHHHH

SEQ ID NO: 5 - protein, 230 aa, Artificial Sequence
  Synthetic sequence
MSQAIGILELRSIAAGMELGDAMLKSANVDLLVSKTISRGKFLLMLGGDIGAIQQAIETGTSQAGRLLVDSLVLANIHPSVLPAISGLNSVDCRQAVGIVETRSVAACISAADRAVKGSNVTLVRVHMARGIGGKCYMVVAGDVSDVALAVTVASSSAGAYGRLVYASLIPRPHEAMWRQMVEGLEHHHHHHEFPPEVEEQDDGTLPMSCAQESGMDRHPAACASARINV

SEQ ID NO: 6 - protein, 192 aa, Artificial Sequence
  Synthetic sequence
MSQAIGILELTSIAAGMELGDAMLKSANVDLLVSKTISRGKFLLMLGGDIGAIQQAIETGTSQAGELLVDSLVLANIHPSVLPAISGLNSVDKRQAVGIVETWSVAACISAADRAVKGSNVTLVRVHMAFGIGGKCYMVVAGDVSDVALAVTVASSSAGAYGLLVYASLIPRPHEAMWRQMVEGLEHHHHHH

SEQ ID NO: 7 - protein, 192 aa, Artificial Sequence
  Synthetic sequence
MSQAIGILELTSIAAGMELGDAMLKSANVDLLVSKTISRGKFLLMLGGDIGAIQQAIETGTSQAGELLVDSLVLANIHPSVLPAISGLNSVDKRQAVGIVETWSVAACISAADRAVKGSNVTLVRVHMARGIGGKCYMVVAGDVSDVALAVTVASSSAGAYGLLVYASLIPRPHEAMWRQMVEGLEHHHHHH

SEQ ID NO: 8 - protein, 192 aa, Artificial Sequence
  Synthetic sequence
MSQAIGILELRSIAAGMELGDAMLKSANVDLLVSKTISPGKFLLMLGGDIGAIQQAIETGTSQAGELLVDSLVLANIHPSVLPAISGLNSVDKRQAVGIVETRSVAACISAADRAVKGSNVTLVRVHMAFGIGGKCYMVVAGDVSDVALAVTVASSSAGAYGLLVYASLIPRPHEAMWRQMVEGLEHHHHHH

SEQ ID NO: 9 - protein, 192 aa, Artificial Sequence
  Synthetic sequence
MSQAIGILELRSIAAGMELGDAMLKSANVDLLVSKTISRGKFLLMLGGDIGAIQQAIETGTSQAGELLVDSLVLANIHPSVLPAISGLNSVDKRQAVGIVETWSVAACISAADRAVKGSNVTLVRVHMAFGIGGKCYMVVAGDVSDVALAVTVASSSAGAYGLLVYASLIPRPHEAMWRQMVEGLEHHHHHH

SEQ ID NO: 10 - protein, 192 aa, Artificial Sequence
  Synthetic sequence
MSQAIGILELTSIAAGMELGDAMLKSANVDLLVSKTISPGKFLLMLGGDIGAIQQAIETGTSQAGELLVDSLVLANIHPSVLPAISGLNSVDKRQAVGIVETRSVAACISAADRAVKGSNVTLVRVHMARGIGGKCYMVVAGDVSDVALAVTVASSSAGAYGRLVYASLIPRPHEAMWRQMVEGLEHHHHHH

SEQ ID NO: 11 - protein, 191 aa, Artificial Sequence
  Synthetic sequence
MSQAIGILELRSIAAGMELGDAMLKSANVDLLVSKTISRGKFLLMLGGDIGAIQQAIETGTSQAGELLVDSLVLANIHPSVLPAISGLNSVDKRQAVGIVETWSVAACISAADRAVKGSNVTLVRVHMARGIGGKCYMVVAGDVSDVALAVTVASSSAGAYGLLVYASLIPRPHEAMWRQMVEGLEHHHHH

SEQ ID NO: 12 - protein, 192 aa, Artificial Sequence
  Synthetic sequence
MSQAIGILELRSIAAGMELGDAMLKSANVDLLVSKTISRGKFLLMLGGDIGAIQQAIETGTSQAGELLVDSLVLANIHPSVLPAISGLNSVDKRQAVGIVETRSVAACISAADRAVKGSNVTLVRVHMARGIGGKCYMVVAGDVSDVALAVTVASSSAGAYGLLVYASLIPRPHEAMWRQMVEGLEHHHHHH

SEQ ID NO: 13 - protein, 192 aa, Artificial Sequence
  Synthetic sequence
MSQAIGILELRSIAAGMELGDAMLKSANVDLLVSKTISPGKFLLMLGGDIGAIQQAIETGTSQAGRLLVDSLVLANIHPSVLPAISGLNSVDKRQAVGIVETRSVAACISAADRAVKGSNVTLVRVHMAFGIGGKCYMVVAGDVSDVALAVTVASSSAGAYGRLVYASLIPRPHEAMWRQMVEGLEHHHHHH

SEQ ID NO: 14 - protein, 192 aa, Artificial Sequence
  Synthetic sequence
MSQAIGILELRSIAAGMELGDAMLKSANVDLLVSKTISPGKFLLMLGGDIGAIQQAIETGTSQAGRLLVDSLVLANIHPSVLPAISGLNSVDKRQAVGIVETRSVAACISAADRAVKGSNVTLVRVHMARGIGGKCYMVVAGDVSDVALAVTVASSSAGAYGRLVYASLIPRPHEAMWRQMVEGLEHHHHHH

SEQ ID NO: 15 - protein, 192 aa, Artificial Sequence
  Synthetic sequence
MSQAIGILELRSIAAGMELGDAMLKSANVDLLVSKTISRGKFLLMLGGDIGAIQQAIETGTSQAGRLLVDSLVLANIHPSVLPAISGLNSVDKRQAVGIVETWSVAACISAADRAVKGSNVTLVRVHMARGIGGKCYMVVAGDVSDVALAVTVASSSAGAYGRLVYASLIPRPHEAMWRQMVEGLEHHHHHH

SEQ ID NO: 16 - protein, 192 aa, Artificial Sequence
  Synthetic sequence
MSQAIGILELRSIAAGMELGDAMLKSANVDLLVSKTISRGKFLLMLGGDIGAIQQAIETGTSQAGRLLVDSLVLANIHPSVLPAISGLNSVDKRQAVGIVETRSVAACISAADRAVKGSNVTLVRVHMARGIGGKCYMVVAGDVSDVALAVTVASSSAGAYGLLVYASLIPRPHEAMWRQMVEGLEHHHHHH

SEQ ID NO: 17 - protein, 38 aa, Artificial Sequence
  Synthetic sequence
EFPPEVEEQDDGTLPMSCAQESGMDRHPAACASARINV

SEQ ID NO: 18 - DNA, 21 bp, Artificial Sequence
  Synthetic sequence
ttaattaaagacttcaagcgg

SEQ ID NO: 19 - DNA, 21 bp, Artificial Sequence
  Synthetic sequence
gcttgaagtctttaattaatt

SEQ ID NO: 20 - protein, 189 aa, Artificial Sequence
  Synthetic sequence
MSQAIGILELRSIAAGMELGDAMLKSANVDLLVSKTISRGKFLLMLGGDIGAIQQAIETGTSQAGRLLVDSLVLANIHPSVLPAISGLNSVDKRQAVGIVETRSVAACISAADRAVKGSNVTLVRVHMARGIGGKCYMVVAGDVSDVALAVTVASSSAGAYGRLVYASLIPRPHEAMWRQMVEGLEHHH

SEQ ID NO: 21 - protein, 195 aa, Artificial Sequence
  Synthetic sequence
MSQAIGILELRSIAAGMELGDAMLKSANVDLLVSKTISRGKFLLMLGGDIGAIQQAIETGTSQAGRLLVDSLVLANIHPSVLPAISGLNSVDKRQAVGIVETRSVAACISAADRAVKGSNVTLVRVHMARGIGGKCYMVVAGDVSDVALAVTVASSSAGAYGRLVYASLIPRPHEAMWRQMVEGLEHHHHHHHHH

SEQ ID NO: 22 - protein, 192 aa, Artificial Sequence
  Synthetic sequence
MSQAIGILELRSIAAGMELGDAMLKSANVDLLVSKTICRGKFLLMLGGDIGAIQQAIETGTSQAGRLLVDSLVLANIHPSVLPAISGLNSVDKRQAVGIVETRSVAACISAADRAVKGSNVTLVRVHMARGIGGKCYMVVAGDVSDVALAVTVASSSAGAYGRLVYASLIPRPHEAMWRQMVEGLEHHHHHH

SEQ ID NO: 23 - protein, 201 aa, Artificial Sequence
  Synthetic sequence
MGARASGSGSSQAIGILELRSIAAGMELGDAMLKSANVDLLVSKTISRGKFLLMLGGDIGAIQQAIETGTSQAGRLLVDSLVLANIHPSVLPAISGLNSVDKRQAIGILETRSVAACISAADRAVKGSNVTLVRVHMARGIGGKCYMVVAGDVSDVALAVTVASSSAGAYGRLVYASLIPRPHEAMWRQMVEGLEHHHHHH

SEQ ID NO: 24 - protein, 225 aa, Artificial Sequence
  Synthetic sequence
MSQAIGILELRSIAAGMELGDAMLKSANVDLLVSKTISRGKFLLMLGGDIGAIQQAIETGTSQAGRLLVDSLVLANIHPSVLPAISGLNSVDKRQAVGIVETRSVAACISAADRAVKGSNVTLVRVHMARGIGGKCYMVVAGDVSDVALAVTVASSSAGAYGRLVYASLIPRPHEAMWRQMVEGLEHHHHHHEFSGESSTAPGTSPSGESSTAPGKLVQSPKGKA

SEQ ID NO: 25 - protein, 258 aa, Artificial Sequence
  Synthetic sequence
MSQAIGILELRSIAAGMELGDAMLKSANVDLLVSKTISRGKFLLMLGGDIGAIQQAIETGTSQAGRLLVDSLVLANIHPSVLPAISGLNSVDKRQAVGIVETRSVAACISAADRAVKGSNVTLVRVHMARGIGGKCYMVVAGDVSDVALAVTVASSSAGAYGRLVYASLIPRPHEAMWRQMVEGLEHHHHHHEFGSGSGGVDNKFNKEMRNAYWEIALLPNLNNQQKRAFIRSLYDDPSQSANLLAEAKKLNDAQAPK

SEQ ID NO: 26 - protein, 258 aa, Artificial Sequence
  Synthetic sequence
MSQAIGILELRSIAAGMELGDAMLKSANVDLLVSKTISRGKFLLMLGGDIGAIQQAIETGTSQAGRLLVDSLVLANIHPSVLPAISGLNSVDKRQAVGIVETRSVAACISAADRAVKGSNVTLVRVHMARGIGGKCYMVVAGDVSDVALAVTVASSSAGAYGRLVYASLIPRPHEAMWRQMVEGLEHHHHHHEFGSGSGGVDNKFNKEMWAAWEEIRNLPNLNGWQMTAFIASLVDDPSQSANLLAEAKKLNDAQAPK

SEQ ID NO: 27 - protein, 219 aa, Artificial Sequence
  Synthetic sequence
MSQAIGILELRSIAAGMELGDAMLKSANVDLLVSKTISRGKFLLMLGGDIGAIQQAIETGTSQAGRLLVDSLVLANIHPSVLPAISGLNSVDKRQAVGIVETRSVAACISAADRAVKGSNVTLVRVHMARGIGGKCYMVVAGDVSDVALAVTVASSSAGAYGRLVYASLIPRPHEAMWRQMVEGLEHHHHHHEFGSGSGGGGSGGGSSFSIIHTPILPL